European Patent Application EP 4 201 484 A1, published June 28, 2023. Title: Antisense nucleic acids for inducing exon skipping of angiotensin converting enzyme 2 gene. Applicant: KNC Laboratories Co., Ltd. KOBE GAKUIN UVIVERSITY. The sequence listing filed with the application follows.

SEQUENCE LISTING (28 sequences)

SEQ ID NO: 1 - DNA, 195 bp, Homo sapiens
gatgtcccggagccgtatcaatgatgctttccgtctgaatgacaacagcctagagtttctggggatacagccaacacttggacctcctaaccagccccctgtttccatatggctgattgtttttggagttgtgatgggagtgatagtggttggcattgtcatcctgatcttcactgggatcagagatcggaagaa

SEQ ID NO: 2 - DNA, 18 bp, Artificial Sequence
  Antisense oligonucleotide
gctgtatccccagaaact

SEQ ID NO: 3 - DNA, 18 bp, Artificial Sequence
  Antisense oligonucleotide
gatcccagtgaagatcag

SEQ ID NO: 4 - DNA, 18 bp, Artificial Sequence
  Antisense oligonucleotide
tcttccgatctctgatcc

SEQ ID NO: 5 - DNA, 18 bp, Artificial Sequence
  Antisense oligonucleotide
tgatacggctccgggaca

SEQ ID NO: 6 - DNA, 18 bp, Artificial Sequence
  Antisense oligonucleotide
ggctgttgtcattcagac

SEQ ID NO: 7 - DNA, 18 bp, Artificial Sequence
  Antisense oligonucleotide
taggaggtccaagtgttg

SEQ ID NO: 8 - DNA, 18 bp, Artificial Sequence
  Antisense oligonucleotide
ccatatggaaacaggggg

SEQ ID NO: 9 - DNA, 18 bp, Artificial Sequence
  Antisense oligonucleotide
cacaactccaaaaacaat

SEQ ID NO: 10 - DNA, 18 bp, Artificial Sequence
  Antisense oligonucleotide
aatgccaaccactatcac

SEQ ID NO: 11 - DNA, 18 bp, Artificial Sequence
  Antisense oligonucleotide
cgggacatcctatttgca

SEQ ID NO: 12 - DNA, 18 bp, Artificial Sequence
  Antisense oligonucleotide
gccacttacttcttccga

SEQ ID NO: 13 - DNA, 18 bp, Artificial Sequence
  Antisense oligonucleotide
cggctccgggacatccta

SEQ ID NO: 14 - DNA, 18 bp, Artificial Sequence
  Antisense oligonucleotide
cggaaagcatcattgata

SEQ ID NO: 15 - DNA, 18 bp, Artificial Sequence
  Antisense oligonucleotide
ctctaggctgttgtcatt

SEQ ID NO: 16 - DNA, 18 bp, Artificial Sequence
  Antisense oligonucleotide
tccaagtgttggctgtat

SEQ ID NO: 17 - DNA, 18 bp, Artificial Sequence
  Antisense oligonucleotide
agggggctggttaggagg

SEQ ID NO: 18 - DNA, 20 bp, Artificial Sequence
  Primer
ctgttccgatcatctgttgc

SEQ ID NO: 19 - DNA, 22 bp, Artificial Sequence
  Primer
gagaccaaatacacactttccc

SEQ ID NO: 20 - DNA, 18 bp, Artificial Sequence
  Primer
cccttcattgacctcaac

SEQ ID NO: 21 - DNA, 18 bp, Artificial Sequence
  Primer
ttcacacccatgacgaac

SEQ ID NO: 22 - DNA, 18 bp, Artificial Sequence
  Antisense oligonucleotide
ttgtcattcagacggaaa

SEQ ID NO: 23 - DNA, 18 bp, Artificial Sequence
  Antisense oligonucleotide
tgtcattcagacggaaag

SEQ ID NO: 24 - DNA, 18 bp, Artificial Sequence
  Antisense oligonucleotide
gtcattcagacggaaagc

SEQ ID NO: 25 - DNA, 18 bp, Artificial Sequence
  Antisense oligonucleotide
tcattcagacggaaagca

SEQ ID NO: 26 - DNA, 18 bp, Artificial Sequence
  Antisense oligonuleotide
attcagacggaaagcatc

SEQ ID NO: 27 - DNA, 18 bp, Artificial Sequence
  Antisense Oligonucleotdie
tcagacggaaagcatcat

SEQ ID NO: 28 - DNA, 18 bp, Artificial Sequence
  Antisense oligonucleotide
ggctgttgtcattcagac